European Patent Application EP 4 335 919 A1, published March 13, 2024. Title: Culture method of dendritic cells. Applicant: NANOFAENTECH CO., Ltd. AJOU UNIVERSITY INDUSTRY-ACADEMIC COOPERATION FOUNDATION. The sequence listing filed with the application follows.

SEQUENCE LISTING (23 sequences)

SEQ ID NO: 1 - protein, 3 aa, Artificial Sequence
  Fibronectin motif P1
RGD

SEQ ID NO: 2 - protein, 3 aa, Artificial Sequence
  Fibronectin motif P2
LDV

SEQ ID NO: 3 - protein, 5 aa, Artificial Sequence
  Fibronectin motif P3
PHSRN

SEQ ID NO: 4 - protein, 6 aa, Artificial Sequence
  Fibronectin motif like peptide P1-1
KGRGDS

SEQ ID NO: 5 - protein, 5 aa, Artificial Sequence
  Fibronectin motif like peptide P1-2
GRGDS

SEQ ID NO: 6 - protein, 11 aa, Artificial Sequence
  Fibronectin motif like peptide P2-1
GGPEILDVPST

SEQ ID NO: 7 - protein, 8 aa, Artificial Sequence
  Fibronectin motif like peptide P2-2
EILDVPST

SEQ ID NO: 8 - protein, 2 aa, Artificial Sequence
  Linker
GS

SEQ ID NO: 9 - protein, 4 aa, Artificial Sequence
  Linker
GGGS

SEQ ID NO: 10 - protein, 5 aa, Artificial Sequence
  Linker
GGGGS

SEQ ID NO: 11 - protein, 8 aa, Artificial Sequence
  Linker
GGGSGGGS

SEQ ID NO: 12 - protein, 15 aa, Artificial Sequence
  Linker peptide LP1
PHSRNGSRGDGSLDV

SEQ ID NO: 13 - protein, 19 aa, Artificial Sequence
  Linker peptide LP2
PHSRNGGGSRGDGGGSLDV

SEQ ID NO: 14 - protein, 23 aa, Artificial Sequence
  Linker peptide LP3
PHSRNGGGSGGGSRGDGGGSLDV

SEQ ID NO: 15 - protein, 3 aa, Artificial Sequence
  Scrambled motif S-P1
GDR

SEQ ID NO: 16 - protein, 3 aa, Artificial Sequence
  Scrambled motif S-P2
VLD

SEQ ID NO: 17 - protein, 5 aa, Artificial Sequence
  Scrambled motif S-P3
SNPRH

SEQ ID NO: 18 - protein, 6 aa, Artificial Sequence
  Laminin derived peptide P4
  MISC_FEATURE (3): Xaa means Hyp(hydroxyproline)
GFXGER

SEQ ID NO: 19 - protein, 5 aa, Artificial Sequence
  Laminin derived peptide P5
YIGSR

SEQ ID NO: 20 - protein, 5 aa, Artificial Sequence
  Laminin derived peptide P6
IKVAV

SEQ ID NO: 21 - protein, 15 aa, Artificial Sequence
  Scrambled linker peptide S-LP1
NRPHSGSDRGGSVDL

SEQ ID NO: 22 - protein, 19 aa, Artificial Sequence
  Scrambled linker peptide S-LP2
NRPHSGGGSDRGGGGSVDL

SEQ ID NO: 23 - protein, 23 aa, Artificial Sequence
  Scrambled linker peptide S-LP3
NRPHSGGGSGGGSDRGGGGSVDL